European Patent Specification EP 3 661 967 B1, published October 9, 2024. Title: A RECOMBINANT FLAVIN-ADENINE DINUCLEOTIDE GLUCOSE DEHYDROGENASE AND USES THEREOF. Applicant: B. G. NEGEV TECHNOLOGIES AND APPLICATIONS LTD., AT BEN-GURION UNIVERSITY. The sequence listing filed with the application follows.

SEQUENCE LISTING (26 sequences)

SEQ ID NO: 1 - DNA, 1617 bp, Artificial
  Synthetic
atggcggatacggatacccagaaagcggacgtggtcgtggttggatccggcgtggcaggcgcaatcgtggctcatcaactggcaatggcaggtaaaagcgtgatcctgctggaagctggtccgcgtatgccgcgttgggaaattgttgaacgtttccgcaatcaagtcgataaaaccgactttatggcaccgtatccgagcagcgcatgggcaccgcatccggaatatggtccgccgaatgattacctgatcctgaaaggcgaacacaaatttaactcacagtacattcgtgcagtgggcggcaccacgtggcattgggcagcctcggcatggcgcttcatcccgaacgattttaaaatgaaaaccgtgtatggcgttggtcgtgactggccgattcagtacgatgacatcgaacattattaccaacgcgcggaagaagaactgggcgtgtggggtccgggcccggaagaagacctgtattcaccgcgtaaagaaccgtacccgatgccgccgctgccgctgagtttcaatgaacaaaccattaaatccgctctgaacggctatgatccgaaatttcacgtggttacggaaccggtggcccgtaattcgcgcccgtacgacggtcgcccgacctgctgtggcaacaataactgcatgccgatttgtccgatcggtgcaatgtataacggcatcgtccatgtggaaaaagctgaacaggcaggtgctaaactgattgatagtgcggtcgtgtacaaactggaaacgggcccggacaaacgtattaccgcagctgtttataaagataaaacgggtgcggaccatcgcgtcgaaggcaaatacttcgtgattgcggccaatggtatcgaaaccccgaaaattctgctgatgagcgcgaaccgtgattttccgaatggtgtggccaacagttccgatatggttggccgcaatctgatggaccatccgggcaccggcgtgagcttttatgcaaacgaaaaactgtggccgggtcgtggtccgcaggaaatgacctctctgatcggtttccgtgatggcccgtttcgcgcgaatgaagcagcgaagaaaattcatctgtcaaatatgtcgcgtatcaaccaggaaacccaaaaaatctttaaaggcggtaaactgatgaaaccggaagaactggatgcgcagatccgtgaccgcagtgcccgctttgttcaattcgattgctttcacgaaatcctgccgcagccggaaaatcgtattgtcccgtccaaaaccgcaacggacgcagtgggtattccgcgtccggaaattacgtatgcgatcgatgactacgtcaaacgtggcgcagtgcatacgcgcgaagtttatgctaccgcggccaaagtgctgggcggcaccgaagtggtcttcaacgatgaatttgcgccgaataaccacatcaccggtgccacgattatgggcgcggatgcccgtgactcagtggttgataaagactgtcgcgccttcgatcatccgaacctgtttattagcagcagcagcaccatgccgacggttggcaccgttaacgtcaccctgacgattgcagctctggcactgcgtatgtctgatacgctgaaaaaagaagtc

SEQ ID NO: 2 - DNA, 510 bp, Artificial
  Synthetic
atggctcacaatgacaacaccccgcactcccgccgtaccggcgatgcggccgtgaccggtattacgcgtcgccagtggctgcaaggcgcgctggccctgaccgcagctggcctgacgggttccctggccctgcgcgcactggctgatgatccgggcaccgcaccgctggatacctttatgacgctgagcgaagctctgacgggcaaaaaaggtctgtctcgtgttctgggccagcgttttctgcaagcgctgcaaaaaggttcattcaaaaccgcggattcgctgccgcagctggcgggcgccctggcaagcggttctctgaacccggaccaagaagctctggcgctgaaaatcctggaagcatggtatctgggcattgttgataatgtggttatcacctacgaagaagccctgatgtttagtgtcgtgtccgacacgctggtcattccgagctattgcccgaacaaaccgggtttctgggccgaaaaaccgatcgaacgtcaggcataa

SEQ ID NO: 3 - DNA, 69 bp, Artificial
  Synthetic
attcgtgcaggtgctaccatgccgcatcgtgatcgtggtccgtgcggtgcatgtcacgctattatccag

SEQ ID NO: 4 - DNA, 39 bp, Artificial
  Synthetic
gaattcggttctggttatggctctggtccgccgggtccg

SEQ ID NO: 5 - DNA, 2191 bp, Artificial
  Synthetic
ctcacaatgacaacaccccgcactcccgccgtaccggcgatgcggccgtgaccggtattacgcgtcgccagtggctgcaaggcgcgctggccctgaccgcagctggcctgacgggttccctggccctgcgcgcactggctgatgatccgggcaccgcaccgctggatacctttatgacgctgagcgaagctctgacgggcaaaaaaggtctgtctcgtgttctgggccagcgttttctgcaagcgctgcaaaaaggttcattcaaaaccgcggattcgctgccgcagctggcgggcgccctggcaagcggttctctgaacccggaccaagaagctctggcgctgaaaatcctggaagcatggtatctgggcattgttgataatgtggttatcacctacgaagaagccctgatgtttagtgtcgtgtccgacacgctggtcattccgagctattgcccgaacaaaccgggtttctgggccgaaaaaccgatcgaacgtcaggcataatggcggatacggatacccagaaagcggacgtggtcgtggttggatccggcgtggcaggcgcaatcgtggctcatcaactggcaatggcaggtaaaagcgtgatcctgctggaagctggtccgcgtatgccgcgttgggaaattgttgaacgtttccgcaatcaagtcgataaaaccgactttatggcaccgtatccgagcagcgcatgggcaccgcatccggaatatggtccgccgaatgattacctgatcctgaaaggcgaacacaaatttaactcacagtacattcgtgcagtgggcggcaccacgtggcattgggcagcctcggcatggcgcttcatcccgaacgattttaaaatgaaaaccgtgtatggcgttggtcgtgactggccgattcagtacgatgacatcgaacattattaccaacgcgcggaagaagaactgggcgtgtggggtccgggcccggaagaagacctgtattcaccgcgtaaagaaccgtacccgatgccgccgctgccgctgagtttcaatgaacaaaccattaaatccgctctgaacggctatgatccgaaatttcacgtggttacggaaccggtggcccgtaattcgcgcccgtacgacggtcgcccgacctgctgtggcaacaataactgcatgccgatttgtccgatcggtgcaatgtataacggcatcgtccatgtggaaaaagctgaacaggcaggtgctaaactgattgatagtgcggtcgtgtacaaactggaaacgggcccggacaaacgtattaccgcagctgtttataaagataaaacgggtgcggaccatcgcgtcgaaggcaaatacttcgtgattgcggccaatggtatcgaaaccccgaaaattctgctgatgagcgcgaaccgtgattttccgaatggtgtggccaacagttccgatatggttggccgcaatctgatggaccatccgggcaccggcgtgagcttttatgcaaacgaaaaactgtggccgggtcgtggtccgcaggaaatgacctctctgatcggtttccgtgatggcccgtttcgcgcgaatgaagcagcgaagaaaattcatctgtcaaatatgtcgcgtatcaaccaggaaacccaaaaaatctttaaaggcggtaaactgatgaaaccggaagaactggatgcgcagatccgtgaccgcagtgcccgctttgttcaattcgattgctttcacgaaatcctgccgcagccggaaaatcgtattgtcccgtccaaaaccgcaacggacgcagtgggtattccgcgtccggaaattacgtatgcgatcgatgactacgtcaaacgtggcgcagtgcatacgcgcgaagtttatgctaccgcggccaaagtgctgggcggcaccgaagtggtcttcaacgatgaatttgcgccgaataaccacatcaccggtgccacgattatgggcgcggatgcccgtgactcagtggttgataaagactgtcgcgccttcgatcatccgaacctgtttattagcagcagcagcaccatgccgacggttggcaccgttaacgtcaccctgacgattgcagctctggcactgcgtatgtctgatacgctgaaaaaagaagtcattcgtgcaggtgctaccatgccgcatcgtgatcgtggtccgtgcggtgcatgtcacgctattatccag

SEQ ID NO: 6 - DNA, 2230 bp, Artificial
  Synthetic
ctcacaatgacaacaccccgcactcccgccgtaccggcgatgcggccgtgaccggtattacgcgtcgccagtggctgcaaggcgcgctggccctgaccgcagctggcctgacgggttccctggccctgcgcgcactggctgatgatccgggcaccgcaccgctggatacctttatgacgctgagcgaagctctgacgggcaaaaaaggtctgtctcgtgttctgggccagcgttttctgcaagcgctgcaaaaaggttcattcaaaaccgcggattcgctgccgcagctggcgggcgccctggcaagcggttctctgaacccggaccaagaagctctggcgctgaaaatcctggaagcatggtatctgggcattgttgataatgtggttatcacctacgaagaagccctgatgtttagtgtcgtgtccgacacgctggtcattccgagctattgcccgaacaaaccgggtttctgggccgaaaaaccgatcgaacgtcaggcataatggcggatacggatacccagaaagcggacgtggtcgtggttggatccggcgtggcaggcgcaatcgtggctcatcaactggcaatggcaggtaaaagcgtgatcctgctggaagctggtccgcgtatgccgcgttgggaaattgttgaacgtttccgcaatcaagtcgataaaaccgactttatggcaccgtatccgagcagcgcatgggcaccgcatccggaatatggtccgccgaatgattacctgatcctgaaaggcgaacacaaatttaactcacagtacattcgtgcagtgggcggcaccacgtggcattgggcagcctcggcatggcgcttcatcccgaacgattttaaaatgaaaaccgtgtatggcgttggtcgtgactggccgattcagtacgatgacatcgaacattattaccaacgcgcggaagaagaactgggcgtgtggggtccgggcccggaagaagacctgtattcaccgcgtaaagaaccgtacccgatgccgccgctgccgctgagtttcaatgaacaaaccattaaatccgctctgaacggctatgatccgaaatttcacgtggttacggaaccggtggcccgtaattcgcgcccgtacgacggtcgcccgacctgctgtggcaacaataactgcatgccgatttgtccgatcggtgcaatgtataacggcatcgtccatgtggaaaaagctgaacaggcaggtgctaaactgattgatagtgcggtcgtgtacaaactggaaacgggcccggacaaacgtattaccgcagctgtttataaagataaaacgggtgcggaccatcgcgtcgaaggcaaatacttcgtgattgcggccaatggtatcgaaaccccgaaaattctgctgatgagcgcgaaccgtgattttccgaatggtgtggccaacagttccgatatggttggccgcaatctgatggaccatccgggcaccggcgtgagcttttatgcaaacgaaaaactgtggccgggtcgtggtccgcaggaaatgacctctctgatcggtttccgtgatggcccgtttcgcgcgaatgaagcagcgaagaaaattcatctgtcaaatatgtcgcgtatcaaccaggaaacccaaaaaatctttaaaggcggtaaactgatgaaaccggaagaactggatgcgcagatccgtgaccgcagtgcccgctttgttcaattcgattgctttcacgaaatcctgccgcagccggaaaatcgtattgtcccgtccaaaaccgcaacggacgcagtgggtattccgcgtccggaaattacgtatgcgatcgatgactacgtcaaacgtggcgcagtgcatacgcgcgaagtttatgctaccgcggccaaagtgctgggcggcaccgaagtggtcttcaacgatgaatttgcgccgaataaccacatcaccggtgccacgattatgggcgcggatgcccgtgactcagtggttgataaagactgtcgcgccttcgatcatccgaacctgtttattagcagcagcagcaccatgccgacggttggcaccgttaacgtcaccctgacgattgcagctctggcactgcgtatgtctgatacgctgaaaaaagaagtcgaattcggttctggttatggctctggtccgccgggtccgattcgtgcaggtgctaccatgccgcatcgtgatcgtggtccgtgcggtgcatgtcacgctattatccag

SEQ ID NO: 7 - DNA, 2278 bp, Artificial
  Synthetic
ccatggctcacaatgacaacaccccgcactcccgccgtaccggcgatgcggccgtgaccggtattacgcgtcgccagtggctgcaaggcgcgctggccctgaccgcagctggcctgacgggttccctggccctgcgcgcactggctgatgatccgggcaccgcaccgctggatacctttatgacgctgagcgaagctctgacgggcaaaaaaggtctgtctcgtgttctgggccagcgttttctgcaagcgctgcaaaaaggttcattcaaaaccgcggattcgctgccgcagctggcgggcgccctggcaagcggttctctgaacccggaccaagaagctctggcgctgaaaatcctggaagcatggtatctgggcattgttgataatgtggttatcacctacgaagaagccctgatgtttagtgtcgtgtccgacacgctggtcattccgagctattgcccgaacaaaccgggtttctgggccgaaaaaccgatcgaacgtcaggcataatggcggatacggatacccagaaagcggacgtggtcgtggttggatccggcgtggcaggcgcaatcgtggctcatcaactggcaatggcaggtaaaagcgtgatcctgctggaagctggtccgcgtatgccgcgttgggaaattgttgaacgtttccgcaatcaagtcgataaaaccgactttatggcaccgtatccgagcagcgcatgggcaccgcatccggaatatggtccgccgaatgattacctgatcctgaaaggcgaacacaaatttaactcacagtacattcgtgcagtgggcggcaccacgtggcattgggcagcctcggcatggcgcttcatcccgaacgattttaaaatgaaaaccgtgtatggcgttggtcgtgactggccgattcagtacgatgacatcgaacattattaccaacgcgcggaagaagaactgggcgtgtggggtccgggcccggaagaagacctgtattcaccgcgtaaagaaccgtacccgatgccgccgctgccgctgagtttcaatgaacaaaccattaaatccgctctgaacggctatgatccgaaatttcacgtggttacggaaccggtggcccgtaattcgcgcccgtacgacggtcgcccgacctgctgtggcaacaataactgcatgccgatttgtccgatcggtgcaatgtataacggcatcgtccatgtggaaaaagctgaacaggcaggtgctaaactgattgatagtgcggtcgtgtacaaactggaaacgggcccggacaaacgtattaccgcagctgtttataaagataaaacgggtgcggaccatcgcgtcgaaggcaaatacttcgtgattgcggccaatggtatcgaaaccccgaaaattctgctgatgagcgcgaaccgtgattttccgaatggtgtggccaacagttccgatatggttggccgcaatctgatggaccatccgggcaccggcgtgagcttttatgcaaacgaaaaactgtggccgggtcgtggtccgcaggaaatgacctctctgatcggtttccgtgatggcccgtttcgcgcgaatgaagcagcgaagaaaattcatctgtcaaatatgtcgcgtatcaaccaggaaacccaaaaaatctttaaaggcggtaaactgatgaaaccggaagaactggatgcgcagatccgtgaccgcagtgcccgctttgttcaattcgattgctttcacgaaatcctgccgcagccggaaaatcgtattgtcccgtccaaaaccgcaacggacgcagtgggtattccgcgtccggaaattacgtatgcgatcgatgactacgtcaaacgtggcgcagtgcatacgcgcgaagtttatgctaccgcggccaaagtgctgggcggcaccgaagtggtcttcaacgatgaatttgcgccgaataaccacatcaccggtgccacgattatgggcgcggatgcccgtgactcagtggttgataaagactgtcgcgccttcgatcatccgaacctgtttattagcagcagcagcaccatgccgacggttggcaccgttaacgtcaccctgacgattgcagctctggcactgcgtatgtctgatacgctgaaaaaagaagtcgaattcggttctggttatggctctggtccgccgggtccgattcgtgcaggtgctaccatgccgcatcgtgatcgtggtccgtgcggtgcatgtcacgctattatccagggcagtggttccggccatcaccatcaccatcactaaaagctt

SEQ ID NO: 8 - protein, 527 aa, Artificial
  Synthetic
MADTDTQKADVVVVGSGVAGAIVAHQLAMAGKSVILLEAGPRMPRWEIVERFRNQVDKTDFMAPYPSSAWAPHPEYGPPNDYLILKGEHKFNSQYIRAVGGTTWHWAASAWRFIPNDFKMKTVYGVGRDWPIQYDDIEHYYQRAEEELGVWGPGPEEDLYSPRKEPYPMPPLPLSFNEQTIKSALNGYDPKFHVVTEPVARNSRPYDGRPTCCGNNNCMPICPIGAMYNGIVHVEKAEQAGAKLIDSAVVYKLETGPDKRITAAVYKDKTGADHRVEGKYFVIAANGIETPKILLMSANRDFPNGVANSSDMVGRNLMDHPGTGVSFYANEKLWPGRGPQEMTSLIGFRDGPFRANEAAKKIHLSNMSRINQETQKIFKGGKLMKPEELDAQIRDRSARFVQFDCFHEILPQPENRIVPSKTATDAVGIPRPEITYAIDDYVKRGAVHTREVYATAAKVLGGTEVVFNDEFAPNNHITGATIMGADARDSVVDKDCRAFDHPNLFISSSSTMPTVGTVNVTLTIAAL

SEQ ID NO: 9 - protein, 562 aa, Artificial
  Synthetic
MADTDTQKADVVVVGSGVAGAIVAHQLAMAGKSVILLEAGPRMPRWEIVERFRNQVDKTDFMAPYPSSAWAPHPEYGPPNDYLILKGEHKFNSQYIRAVGGTTWHWAASAWRFIPNDFKMKTVYGVGRDWPIQYDDIEHYYQRAEEELGVWGPGPEEDLYSPRKEPYPMPPLPLSFNEQTIKSALNGYDPKFHVVTEPVARNSRPYDGRPTCCGNNNCMPICPIGAMYNGIVHVEKAEQAGAKLIDSAVVYKLETGPDKRITAAVYKDKTGADHRVEGKYFVIAANGIETPKILLMSANRDFPNGVANSSDMVGRNLMDHPGTGVSFYANEKLWPGRGPQEMTSLIGFRDGPFRANEAAKKIHLSNMSRINQETQKIFKGGKLMKPEELDAQIRDRSARFVQFDCFHEILPQPENRIVPSKTATDAVGIPRPEITYAIDDYVKRGAVHTREVYATAAKVLGGTEVVFNDEFAPNNHITGATIMGADARDSVVDKDCRAFDHPNLFISSSSTMPTVGTVNVTLTIAALALRMSDTLKKEVIRAGATMPHRDRGPCGACHAIIQ

SEQ ID NO: 10 - protein, 586 aa, Artificial
  Synthetic
MADTDTQKADVVVVGSGVAGAIVAHQLAMAGKSVILLEAGPRMPRWEIVERFRNQVDKTDFMAPYPSSAWAPHPEYGPPNDYLILKGEHKFNSQYIRAVGGTTWHWAASAWRFIPNDFKMKTVYGVGRDWPIQYDDIEHYYQRAEEELGVWGPGPEEDLYSPRKEPYPMPPLPLSFNEQTIKSALNGYDPKFHVVTEPVARNSRPYDGRPTCCGNNNCMPICPIGAMYNGIVHVEKAEQAGAKLIDSAVVYKLETGPDKRITAAVYKDKTGADHRVEGKYFVIAANGIETPKILLMSANRDFPNGVANSSDMVGRNLMDHPGTGVSFYANEKLWPGRGPQEMTSLIGFRDGPFRANEAAKKIHLSNMSRINQETQKIFKGGKLMKPEELDAQIRDRSARFVQFDCFHEILPQPENRIVPSKTATDAVGIPRPEITYAIDDYVKRGAVHTREVYATAAKVLGGTEVVFNDEFAPNNHITGATIMGADARDSVVDKDCRAFDHPNLFISSSSTMPTVGTVNVTLTIAALALRMSDTLKKEVEFGSGYGSGPPGPIRAGATMPHRDRGPCGACHAIIQGSGSGHHHHHH

SEQ ID NO: 11 - protein, 575 aa, Artificial
  Synthetic
MADTDTQKADVVVVGSGVAGAIVAHQLAMAGKSVILLEAGPRMPRWEIVERFRNQVDKTDFMAPYPSSAWAPHPEYGPPNDYLILKGEHKFNSQYIRAVGGTTWHWAASAWRFIPNDFKMKTVYGVGRDWPIQYDDIEHYYQRAEEELGVWGPGPEEDLYSPRKEPYPMPPLPLSFNEQTIKSALNGYDPKFHVVTEPVARNSRPYDGRPTCCGNNNCMPICPIGAMYNGIVHVEKAEQAGAKLIDSAVVYKLETGPDKRITAAVYKDKTGADHRVEGKYFVIAANGIETPKILLMSANRDFPNGVANSSDMVGRNLMDHPGTGVSFYANEKLWPGRGPQEMTSLIGFRDGPFRANEAAKKIHLSNMSRINQETQKIFKGGKLMKPEELDAQIRDRSARFVQFDCFHEILPQPENRIVPSKTATDAVGIPRPEITYAIDDYVKRGAVHTREVYATAAKVLGGTEVVFNDEFAPNNHITGATIMGADARDSVVDKDCRAFDHPNLFISSSSTMPTVGTVNVTLTIAALALRMSDTLKKEVEFGSGYGSGPPGPIRAGATMPHRDRGPCGACHAIIQ

SEQ ID NO: 12 - protein, 586 aa, Artificial
  Synthetic
  X (42)..(42): X is R or a non-canonical amino acid.
  X (247)..(247): X is S or a non-canonical amino acid.
  X (395)..(395): X is D or a non-canonical amino acid.
  X (558)..(558): X is T or a non-canonical amino acid.
  X (560)..(560): X is P or a non-canonical amino acid.
MADTDTQKADVVVVGSGVAGAIVAHQLAMAGKSVILLEAGPXMPRWEIVERFRNQVDKTDFMAPYPSSAWAPHPEYGPPNDYLILKGEHKFNSQYIRAVGGTTWHWAASAWRFIPNDFKMKTVYGVGRDWPIQYDDIEHYYQRAEEELGVWGPGPEEDLYSPRKEPYPMPPLPLSFNEQTIKSALNGYDPKFHVVTEPVARNSRPYDGRPTCCGNNNCMPICPIGAMYNGIVHVEKAEQAGAKLIDXAVVYKLETGPDKRITAAVYKDKTGADHRVEGKYFVIAANGIETPKILLMSANRDFPNGVANSSDMVGRNLMDHPGTGVSFYANEKLWPGRGPQEMTSLIGFRDGPFRANEAAKKIHLSNMSRINQETQKIFKGGKLMKPEELDAQIRXRSARFVQFDCFHEILPQPENRIVPSKTATDAVGIPRPEITYAIDDYVKRGAVHTREVYATAAKVLGGTEVVFNDEFAPNNHITGATIMGADARDSVVDKDCRAFDHPNLFISSSSTMPTVGTVNVTLTIAALALRMSDTLKKEVEFGSGYGSGPPGPIRAGAXMXHRDRGPCGACHAIIQGSGSGHHHHHH

SEQ ID NO: 13 - protein, 575 aa, Artificial
  Synthetic
  X (42)..(42): X is R or a non-canonical amino acid
  X (247)..(247): X is S or a non-canonical amino acid
  X (395)..(395): X is D or a non-canonical amino acid
  X (558)..(558): X is T or a non-canonical amino acid
  X (560)..(560): X is P or a non-canonical amino acid
MADTDTQKADVVVVGSGVAGAIVAHQLAMAGKSVILLEAGPXMPRWEIVERFRNQVDKTDFMAPYPSSAWAPHPEYGPPNDYLILKGEHKFNSQYIRAVGGTTWHWAASAWRFIPNDFKMKTVYGVGRDWPIQYDDIEHYYQRAEEELGVWGPGPEEDLYSPRKEPYPMPPLPLSFNEQTIKSALNGYDPKFHVVTEPVARNSRPYDGRPTCCGNNNCMPICPIGAMYNGIVHVEKAEQAGAKLIDXAVVYKLETGPDKRITAAVYKDKTGADHRVEGKYFVIAANGIETPKILLMSANRDFPNGVANSSDMVGRNLMDHPGTGVSFYANEKLWPGRGPQEMTSLIGFRDGPFRANEAAKKIHLSNMSRINQETQKIFKGGKLMKPEELDAQIRXRSARFVQFDCFHEILPQPENRIVPSKTATDAVGIPRPEITYAIDDYVKRGAVHTREVYATAAKVLGGTEVVFNDEFAPNNHITGATIMGADARDSVVDKDCRAFDHPNLFISSSSTMPTVGTVNVTLTIAALALRMSDTLKKEVEFGSGYGSGPPGPIRAGAXMXHRDRGPCGACHAIIQ

SEQ ID NO: 14 - DNA, 1727 bp, Artificial
  Synthetic
tggcggatacggatacccagaaagcggacgtggtcgtggttggatccggcgtggcaggcgcaatcgtggctcatcaactggcaatggcaggtaaaagcgtgatcctgctggaagctggtccgtagatgccgcgttgggaaattgttgaacgtttccgcaatcaagtcgataaaaccgactttatggcaccgtatccgagcagcgcatgggcaccgcatccggaatatggtccgccgaatgattacctgatcctgaaaggcgaacacaaatttaactcacagtacattcgtgcagtgggcggcaccacgtggcattgggcagcctcggcatggcgcttcatcccgaacgattttaaaatgaaaaccgtgtatggcgttggtcgtgactggccgattcagtacgatgacatcgaacattattaccaacgcgcggaagaagaactgggcgtgtggggtccgggcccggaagaagacctgtattcaccgcgtaaagaaccgtacccgatgccgccgctgccgctgagtttcaatgaacaaaccattaaatccgctctgaacggctatgatccgaaatttcacgtggttacggaaccggtggcccgtaattcgcgcccgtacgacggtcgcccgacctgctgtggcaacaataactgcatgccgatttgtccgatcggtgcaatgtataacggcatcgtccatgtggaaaaagctgaacaggcaggtgctaaactgattgatagtgcggtcgtgtacaaactggaaacgggcccggacaaacgtattaccgcagctgtttataaagataaaacgggtgcggaccatcgcgtcgaaggcaaatacttcgtgattgcggccaatggtatcgaaaccccgaaaattctgctgatgagcgcgaaccgtgattttccgaatggtgtggccaacagttccgatatggttggccgcaatctgatggaccatccgggcaccggcgtgagcttttatgcaaacgaaaaactgtggccgggtcgtggtccgcaggaaatgacctctctgatcggtttccgtgatggcccgtttcgcgcgaatgaagcagcgaagaaaattcatctgtcaaatatgtcgcgtatcaaccaggaaacccaaaaaatctttaaaggcggtaaactgatgaaaccggaagaactggatgcgcagatccgtgaccgcagtgcccgctttgttcaattcgattgctttcacgaaatcctgccgcagccggaaaatcgtattgtcccgtccaaaaccgcaacggacgcagtgggtattccgcgtccggaaattacgtatgcgatcgatgactacgtcaaacgtggcgcagtgcatacgcgcgaagtttatgctaccgcggccaaagtgctgggcggcaccgaagtggtcttcaacgatgaatttgcgccgaataaccacatcaccggtgccacgattatgggcgcggatgcccgtgactcagtggttgataaagactgtcgcgccttcgatcatccgaacctgtttattagcagcagcagcaccatgccgacggttggcaccgttaacgtcaccctgacgattgcagctctggcactgcgtatgtctgatacgctgaaaaaagaagtcgaattcggttctggttatggctctggtccgccgggtccgattcgtgcaggtgctaccatgccgcatcgtgatcgtggtccgtgcggtgcatgtcacgctattatccagtaa

SEQ ID NO: 15 - DNA, 1728 bp, Artificial
  Synthetic
atggcggatacggatacccagaaagcggacgtggtcgtggttggatccggcgtggcaggcgcaatcgtggctcatcaactggcaatggcaggtaaaagcgtgatcctgctggaagctggtccgcgtatgccgcgttgggaaattgttgaacgtttccgcaatcaagtcgataaaaccgactttatggcaccgtatccgagcagcgcatgggcaccgcatccggaatatggtccgccgaatgattacctgatcctgaaaggcgaacacaaatttaactcacagtacattcgtgcagtgggcggcaccacgtggcattgggcagcctcggcatggcgcttcatcccgaacgattttaaaatgaaaaccgtgtatggcgttggtcgtgactggccgattcagtacgatgacatcgaacattattaccaacgcgcggaagaagaactgggcgtgtggggtccgggcccggaagaagacctgtattcaccgcgtaaagaaccgtacccgatgccgccgctgccgctgagtttcaatgaacaaaccattaaatccgctctgaacggctatgatccgaaatttcacgtggttacggaaccggtggcccgtaattcgcgcccgtacgacggtcgcccgacctgctgtggcaacaataactgcatgccgatttgtccgatcggtgcaatgtataacggcatcgtccatgtggaaaaagctgaacaggcaggtgctaaactgattgattaggcggtcgtgtacaaactggaaacgggcccggacaaacgtattaccgcagctgtttataaagataaaacgggtgcggaccatcgcgtcgaaggcaaatacttcgtgattgcggccaatggtatcgaaaccccgaaaattctgctgatgagcgcgaaccgtgattttccgaatggtgtggccaacagttccgatatggttggccgcaatctgatggaccatccgggcaccggcgtgagcttttatgcaaacgaaaaactgtggccgggtcgtggtccgcaggaaatgacctctctgatcggtttccgtgatggcccgtttcgcgcgaatgaagcagcgaagaaaattcatctgtcaaatatgtcgcgtatcaaccaggaaacccaaaaaatctttaaaggcggtaaactgatgaaaccggaagaactggatgcgcagatccgtgaccgcagtgcccgctttgttcaattcgattgctttcacgaaatcctgccgcagccggaaaatcgtattgtcccgtccaaaaccgcaacggacgcagtgggtattccgcgtccggaaattacgtatgcgatcgatgactacgtcaaacgtggcgcagtgcatacgcgcgaagtttatgctaccgcggccaaagtgctgggcggcaccgaagtggtcttcaacgatgaatttgcgccgaataaccacatcaccggtgccacgattatgggcgcggatgcccgtgactcagtggttgataaagactgtcgcgccttcgatcatccgaacctgtttattagcagcagcagcaccatgccgacggttggcaccgttaacgtcaccctgacgattgcagctctggcactgcgtatgtctgatacgctgaaaaaagaagtcgaattcggttctggttatggctctggtccgccgggtccgattcgtgcaggtgctaccatgccgcatcgtgatcgtggtccgtgcggtgcatgtcacgctattatccagtaa

SEQ ID NO: 16 - DNA, 1729 bp, Artificial
  Synthetic
atggcggatacggatacccagaaagcggacgtggtcgtggttggatccggcgtggcaggcgcaatcgtggctcatcaactggcaatggcaggtaaaagcgtgatcctgctggaagctggtccgcgtatgccgcgttgggaaattgttgaacgtttccgcaatcaagtcgataaaaccgactttatggcaccgtatccgagcagcgcatgggcaccgcatccggaatatggtccgccgaatgattacctgatcctgaaaggcgaacacaaatttaactcacagtacattcgtgcagtgggcggcaccacgtggcattgggcagcctcggcatggcgcttcatcccgaacgattttaaaatgaaaaccgtgtatggcgttggtcgtgactggccgattcagtacgatgacatcgaacattattaccaacgcgcggaagaagaactgggcgtgtggggtccgggcccggaagaagacctgtattcaccgcgtaaagaaccgtacccgatgccgccgctgccgctgagtttcaatgaacaaaccattaaatccgctctgaacggctatgatccgaaatttcacgtggttacggaaccggtggcccgtaattcgcgcccgtacgacggtcgcccgacctgctgtggcaacaataactgcatgccgatttgtccgatcggtgcaatgtataacggcatcgtccatgtggaaaaagctgaacaggcaggtgctaaactgattgatagtgcggtcgtgtacaaactggaaacgggcccggacaaacgtattaccgcagctgtttataaagataaaacgggtgcggaccatcgcgtcgaaggcaaatacttcgtgattgcggccaatggtatcgaaaccccgaaaattctgctgatgagcgcgaaccgtgattttccgaatggtgtggccaacagttccgatatggttggccgcaatctgatggaccatccgggcaccggcgtgagcttttatgcaaacgaaaaactgtggccgggtcgtggtccgcaggaaatgacctctctgatcggtttccgtgatggcccgtttcgcgcgaatgaagcagcgaagaaaattcatctgtcaaatatgtcgcgtatcaaccaggaaacccaaaaaatctttaaaggcggtaaactgatgaaaccggaagaactggatgcgcagatccgttagcgcagtgcccgctttgttcaattcgattgctttcacgaaatcctgccgcagccggaaaatcgtattgtcccgtccaaaaccgcaacggacgcagtgggtattccgcgtccggaaattacgtatgcgatcgatgactacgtcaaacgtggcgcagtgcatacgcgcgaagtttatgctaccgcggccaaagtgctgggcggcaccgaagtggtcttcaacgatgaatttgcgccgaataaccacatcaccggtgccacgattatgggcgcggatgcccgtgactcagtggttgataaagactgtcgcgccttcgatcatccgaacctgtttattagcagcagcagcaccatgccgacggttggcaccgttaacgtcaccctgacgattgcagctctggcactgcgtatgtctgatacgctgaaaaaagaagtcgaattcggttctggttatggctctggtccgccgggtccgattcgtgcaggtgctaccatgccgcatcgtgatcgtggtccgtgcggtgcatgtcacgctattatccaggtaa

SEQ ID NO: 17 - DNA, 1728 bp, Artificial
  Synthetic
atggcggatacggatacccagaaagcggacgtggtcgtggttggatccggcgtggcaggcgcaatcgtggctcatcaactggcaatggcaggtaaaagcgtgatcctgctggaagctggtccgcgtatgccgcgttgggaaattgttgaacgtttccgcaatcaagtcgataaaaccgactttatggcaccgtatccgagcagcgcatgggcaccgcatccggaatatggtccgccgaatgattacctgatcctgaaaggcgaacacaaatttaactcacagtacattcgtgcagtgggcggcaccacgtggcattgggcagcctcggcatggcgcttcatcccgaacgattttaaaatgaaaaccgtgtatggcgttggtcgtgactggccgattcagtacgatgacatcgaacattattaccaacgcgcggaagaagaactgggcgtgtggggtccgggcccggaagaagacctgtattcaccgcgtaaagaaccgtacccgatgccgccgctgccgctgagtttcaatgaacaaaccattaaatccgctctgaacggctatgatccgaaatttcacgtggttacggaaccggtggcccgtaattcgcgcccgtacgacggtcgcccgacctgctgtggcaacaataactgcatgccgatttgtccgatcggtgcaatgtataacggcatcgtccatgtggaaaaagctgaacaggcaggtgctaaactgattgatagtgcggtcgtgtacaaactggaaacgggcccggacaaacgtattaccgcagctgtttataaagataaaacgggtgcggaccatcgcgtcgaaggcaaatacttcgtgattgcggccaatggtatcgaaaccccgaaaattctgctgatgagcgcgaaccgtgattttccgaatggtgtggccaacagttccgatatggttggccgcaatctgatggaccatccgggcaccggcgtgagcttttatgcaaacgaaaaactgtggccgggtcgtggtccgcaggaaatgacctctctgatcggtttccgtgatggcccgtttcgcgcgaatgaagcagcgaagaaaattcatctgtcaaatatgtcgcgtatcaaccaggaaacccaaaaaatctttaaaggcggtaaactgatgaaaccggaagaactggatgcgcagatccgtgaccgcagtgcccgctttgttcaattcgattgctttcacgaaatcctgccgcagccggaaaatcgtattgtcccgtccaaaaccgcaacggacgcagtgggtattccgcgtccggaaattacgtatgcgatcgatgactacgtcaaacgtggcgcagtgcatacgcgcgaagtttatgctaccgcggccaaagtgctgggcggcaccgaagtggtcttcaacgatgaatttgcgccgaataaccacatcaccggtgccacgattatgggcgcggatgcccgtgactcagtggttgataaagactgtcgcgccttcgatcatccgaacctgtttattagcagcagcagcaccatgccgacggttggcaccgttaacgtcaccctgacgattgcagctctggcactgcgtatgtctgatacgctgaaaaaagaagtcgaattcggttctggttatggctctggtccgccgggtccgattcgtgcaggtgcttagatgccgcatcgtgatcgtggtccgtgcggtgcatgtcacgctattatccagtaa

SEQ ID NO: 18 - DNA, 1728 bp, Artificial
  Synthetic
atggcggatacggatacccagaaagcggacgtggtcgtggttggatccggcgtggcaggcgcaatcgtggctcatcaactggcaatggcaggtaaaagcgtgatcctgctggaagctggtccgcgtatgccgcgttgggaaattgttgaacgtttccgcaatcaagtcgataaaaccgactttatggcaccgtatccgagcagcgcatgggcaccgcatccggaatatggtccgccgaatgattacctgatcctgaaaggcgaacacaaatttaactcacagtacattcgtgcagtgggcggcaccacgtggcattgggcagcctcggcatggcgcttcatcccgaacgattttaaaatgaaaaccgtgtatggcgttggtcgtgactggccgattcagtacgatgacatcgaacattattaccaacgcgcggaagaagaactgggcgtgtggggtccgggcccggaagaagacctgtattcaccgcgtaaagaaccgtacccgatgccgccgctgccgctgagtttcaatgaacaaaccattaaatccgctctgaacggctatgatccgaaatttcacgtggttacggaaccggtggcccgtaattcgcgcccgtacgacggtcgcccgacctgctgtggcaacaataactgcatgccgatttgtccgatcggtgcaatgtataacggcatcgtccatgtggaaaaagctgaacaggcaggtgctaaactgattgatagtgcggtcgtgtacaaactggaaacgggcccggacaaacgtattaccgcagctgtttataaagataaaacgggtgcggaccatcgcgtcgaaggcaaatacttcgtgattgcggccaatggtatcgaaaccccgaaaattctgctgatgagcgcgaaccgtgattttccgaatggtgtggccaacagttccgatatggttggccgcaatctgatggaccatccgggcaccggcgtgagcttttatgcaaacgaaaaactgtggccgggtcgtggtccgcaggaaatgacctctctgatcggtttccgtgatggcccgtttcgcgcgaatgaagcagcgaagaaaattcatctgtcaaatatgtcgcgtatcaaccaggaaacccaaaaaatctttaaaggcggtaaactgatgaaaccggaagaactggatgcgcagatccgtgaccgcagtgcccgctttgttcaattcgattgctttcacgaaatcctgccgcagccggaaaatcgtattgtcccgtccaaaaccgcaacggacgcagtgggtattccgcgtccggaaattacgtatgcgatcgatgactacgtcaaacgtggcgcagtgcatacgcgcgaagtttatgctaccgcggccaaagtgctgggcggcaccgaagtggtcttcaacgatgaatttgcgccgaataaccacatcaccggtgccacgattatgggcgcggatgcccgtgactcagtggttgataaagactgtcgcgccttcgatcatccgaacctgtttattagcagcagcagcaccatgccgacggttggcaccgttaacgtcaccctgacgattgcagctctggcactgcgtatgtctgatacgctgaaaaaagaagtcgaattcggttctggttatggctctggtccgccgggtccgattcgtgcaggtgctaccatgtagcatcgtgatcgtggtccgtgcggtgcatgtcacgctattatccagtaa

SEQ ID NO: 19 - protein, 575 aa, Artificial
  Synthetic
  X (42)..(42): X is a non-canonical amino acid
MADTDTQKADVVVVGSGVAGAIVAHQLAMAGKSVILLEAGPXMPRWEIVERFRNQVDKTDFMAPYPSSAWAPHPEYGPPNDYLILKGEHKFNSQYIRAVGGTTWHWAASAWRFIPNDFKMKTVYGVGRDWPIQYDDIEHYYQRAEEELGVWGPGPEEDLYSPRKEPYPMPPLPLSFNEQTIKSALNGYDPKFHVVTEPVARNSRPYDGRPTCCGNNNCMPICPIGAMYNGIVHVEKAEQAGAKLIDSAVVYKLETGPDKRITAAVYKDKTGADHRVEGKYFVIAANGIETPKILLMSANRDFPNGVANSSDMVGRNLMDHPGTGVSFYANEKLWPGRGPQEMTSLIGFRDGPFRANEAAKKIHLSNMSRINQETQKIFKGGKLMKPEELDAQIRDRSARFVQFDCFHEILPQPENRIVPSKTATDAVGIPRPEITYAIDDYVKRGAVHTREVYATAAKVLGGTEVVFNDEFAPNNHITGATIMGADARDSVVDKDCRAFDHPNLFISSSSTMPTVGTVNVTLTIAALALRMSDTLKKEVEFGSGYGSGPPGPIRAGATMPHRDRGPCGACHAIIQ

SEQ ID NO: 20 - protein, 575 aa, Artificial
  Synthetic
  X (247)..(247): X is a non-canonical amino acid
MADTDTQKADVVVVGSGVAGAIVAHQLAMAGKSVILLEAGPRMPRWEIVERFRNQVDKTDFMAPYPSSAWAPHPEYGPPNDYLILKGEHKFNSQYIRAVGGTTWHWAASAWRFIPNDFKMKTVYGVGRDWPIQYDDIEHYYQRAEEELGVWGPGPEEDLYSPRKEPYPMPPLPLSFNEQTIKSALNGYDPKFHVVTEPVARNSRPYDGRPTCCGNNNCMPICPIGAMYNGIVHVEKAEQAGAKLIDXAVVYKLETGPDKRITAAVYKDKTGADHRVEGKYFVIAANGIETPKILLMSANRDFPNGVANSSDMVGRNLMDHPGTGVSFYANEKLWPGRGPQEMTSLIGFRDGPFRANEAAKKIHLSNMSRINQETQKIFKGGKLMKPEELDAQIRDRSARFVQFDCFHEILPQPENRIVPSKTATDAVGIPRPEITYAIDDYVKRGAVHTREVYATAAKVLGGTEVVFNDEFAPNNHITGATIMGADARDSVVDKDCRAFDHPNLFISSSSTMPTVGTVNVTLTIAALALRMSDTLKKEVEFGSGYGSGPPGPIRAGATMPHRDRGPCGACHAIIQ

SEQ ID NO: 21 - protein, 575 aa, Artificial
  Synthetic
  X (395)..(395): X is a non-canonical amino acid
MADTDTQKADVVVVGSGVAGAIVAHQLAMAGKSVILLEAGPRMPRWEIVERFRNQVDKTDFMAPYPSSAWAPHPEYGPPNDYLILKGEHKFNSQYIRAVGGTTWHWAASAWRFIPNDFKMKTVYGVGRDWPIQYDDIEHYYQRAEEELGVWGPGPEEDLYSPRKEPYPMPPLPLSFNEQTIKSALNGYDPKFHVVTEPVARNSRPYDGRPTCCGNNNCMPICPIGAMYNGIVHVEKAEQAGAKLIDSAVVYKLETGPDKRITAAVYKDKTGADHRVEGKYFVIAANGIETPKILLMSANRDFPNGVANSSDMVGRNLMDHPGTGVSFYANEKLWPGRGPQEMTSLIGFRDGPFRANEAAKKIHLSNMSRINQETQKIFKGGKLMKPEELDAQIRXRSARFVQFDCFHEILPQPENRIVPSKTATDAVGIPRPEITYAIDDYVKRGAVHTREVYATAAKVLGGTEVVFNDEFAPNNHITGATIMGADARDSVVDKDCRAFDHPNLFISSSSTMPTVGTVNVTLTIAALALRMSDTLKKEVEFGSGYGSGPPGPIRAGATMPHRDRGPCGACHAIIQ

SEQ ID NO: 22 - protein, 575 aa, Artificial
  Synthetic
  X (558)..(558): X is a non-canonical amino acid
MADTDTQKADVVVVGSGVAGAIVAHQLAMAGKSVILLEAGPRMPRWEIVERFRNQVDKTDFMAPYPSSAWAPHPEYGPPNDYLILKGEHKFNSQYIRAVGGTTWHWAASAWRFIPNDFKMKTVYGVGRDWPIQYDDIEHYYQRAEEELGVWGPGPEEDLYSPRKEPYPMPPLPLSFNEQTIKSALNGYDPKFHVVTEPVARNSRPYDGRPTCCGNNNCMPICPIGAMYNGIVHVEKAEQAGAKLIDSAVVYKLETGPDKRITAAVYKDKTGADHRVEGKYFVIAANGIETPKILLMSANRDFPNGVANSSDMVGRNLMDHPGTGVSFYANEKLWPGRGPQEMTSLIGFRDGPFRANEAAKKIHLSNMSRINQETQKIFKGGKLMKPEELDAQIRDRSARFVQFDCFHEILPQPENRIVPSKTATDAVGIPRPEITYAIDDYVKRGAVHTREVYATAAKVLGGTEVVFNDEFAPNNHITGATIMGADARDSVVDKDCRAFDHPNLFISSSSTMPTVGTVNVTLTIAALALRMSDTLKKEVEFGSGYGSGPPGPIRAGAXMPHRDRGPCGACHAIIQ

SEQ ID NO: 23 - protein, 575 aa, Artificial
  Synthetic
  X (560)..(560): X is a non-canonical amino acid
MADTDTQKADVVVVGSGVAGAIVAHQLAMAGKSVILLEAGPRMPRWEIVERFRNQVDKTDFMAPYPSSAWAPHPEYGPPNDYLILKGEHKFNSQYIRAVGGTTWHWAASAWRFIPNDFKMKTVYGVGRDWPIQYDDIEHYYQRAEEELGVWGPGPEEDLYSPRKEPYPMPPLPLSFNEQTIKSALNGYDPKFHVVTEPVARNSRPYDGRPTCCGNNNCMPICPIGAMYNGIVHVEKAEQAGAKLIDSAVVYKLETGPDKRITAAVYKDKTGADHRVEGKYFVIAANGIETPKILLMSANRDFPNGVANSSDMVGRNLMDHPGTGVSFYANEKLWPGRGPQEMTSLIGFRDGPFRANEAAKKIHLSNMSRINQETQKIFKGGKLMKPEELDAQIRDRSARFVQFDCFHEILPQPENRIVPSKTATDAVGIPRPEITYAIDDYVKRGAVHTREVYATAAKVLGGTEVVFNDEFAPNNHITGATIMGADARDSVVDKDCRAFDHPNLFISSSSTMPTVGTVNVTLTIAALALRMSDTLKKEVEFGSGYGSGPPGPIRAGATMXHRDRGPCGACHAIIQ

SEQ ID NO: 24 - DNA, 18 bp, Artificial
  Synthetic
catcaccatcaccatcac

SEQ ID NO: 25 - DNA, 15 bp, Artificial
  Synthetic
ggcagtggttccggc

SEQ ID NO: 26 - DNA, 2278 bp, Artificial; identical to SEQ ID NO: 7
  Synthetic